European Patent Application EP 4 183 740 A1, published May 24, 2023. Title: Proceso para la obtención de chips Janus, doble planares suspendidos de SU-8, dichos chips Janus, doble planares suspendidos de SU-8 y su arreglo suspendido. Applicant: CONSEJO SUPERIOR DE INVESTIGACIONES CIENTÍFICAS (CSIC). The sequence listing filed with the application follows.

SEQUENCE LISTING (4 sequences)

SEQ ID NO: 1 - DNA, 19 bp, Secuencia Artificial
  Oligonucleótido TS314
cttggagcgaacgacctac

SEQ ID NO: 2 - DNA, 19 bp, Secuencia Artificial
  Oligonucleótido RP-TS314
gtaggtcgttcgctccaag

SEQ ID NO: 3 - DNA, 20 bp, Secuencia Artificial
  Oligonucleótido TS315
caacactcaaccctatctcg

SEQ ID NO: 4 - DNA, 20 bp, Secuencia Artificial
  Oligonucleótido RP-TS315
cgagatagggttgagtgttg